European Patent Application EP 4 116 423 A1, published January 11, 2023. Title: ポリイソプレノイドの製造方法、ベクター、形質転換植物、空気入りタイヤの製造方法及びゴム製品の製造方法. Applicant: 住友ゴム工業株式会社 SUMITOMO RUBBER INDUSTRIES, LTD. 国立大学法人東北大学 TOHOKU UNIVERSITY 国立大学法人金沢大学 KANAZAWA UNIVERSITY. The sequence listing filed with the application follows.

SEQUENCE LISTING (24 sequences)

SEQ ID NO: 1 - DNA, 912 bp, Solanum lycopersicum
atgagttctttggttcttcaatgttggaaattatcatctccatctctgattttacaacaaaatacatcaatatccatgggtgcattcaaaggtattcataaacttcaaatcccaaattcgcctctgacagtgtctgctcgtggactcaacaagatttcatgctcactcaacttacaaaccgaaaagctttgttatgaggataatgataatgatcttgatgaagaacttatgcctaaacacattgctttgataatggatggtaataggagatgggcaaaggataagggtttagaagtatatgaaggtcacaaacatattattccaaaattaaaagagatttgtgacatttcttctaaattgggaatacaaattatcactgcttttgcattctctactgaaaattggaaacgatccaaggaggaggttgatttcttgttgcaaatgttcgaagaaatctatgatgagttttcgaggtctggagtaagagtgtctattataggttgtaaatccgacctcccaatgacattacaaaaatgcatagcattaacagaagagactacaaagggcaacaaaggacttcaccttgtgattgcactaaactatggtggatattatgacatattgcaagcaacaaaaagcattgttaataaagcaatgaatggtttattagatgtagaagatatcaacaagaatttatttgatcaagaacttgaaagcaagtgtccaaatcctgatttacttataaggacaggaggtgaacaaagagttagtaactttttgttgtggcaattggcttacactgaattttacttcaccaacacattgtttcctgattttggagaggaagatcttaaagaggcaataatgaactttcaacaaaggcatagacgttttggtggacacacatattga

SEQ ID NO: 2 - protein, 303 aa, Solanum lycopersicum
MSSLVLQCWKLSSPSLILQQNTSISMGAFKGIHKLQIPNSPLTVSARGLNKISCSLNLQTEKLCYEDNDNDLDEELMPKHIALIMDGNRRWAKDKGLEVYEGHKHIIPKLKEICDISSKLGIQIITAFAFSTENWKRSKEEVDFLLQMFEEIYDEFSRSGVRVSIIGCKSDLPMTLQKCIALTEETTKGNKGLHLVIALNYGGYYDILQATKSIVNKAMNGLLDVEDINKNLFDQELESKCPNPDLLIRTGGEQRVSNFLLWQLAYTEFYFTNTLFPDFGEEDLKEAIMNFQQRHRRFGGHTY

SEQ ID NO: 3 - DNA, 1650 bp, Hevea brasiliensis
gtagtcacagcataagttggagcaaacacaaaactacaggcctcccaggttttaaaaaaaaaaaaaaacttttctacgcataaattttccaagaaaaatatttttgaggaataatttatttttattgttctgttaaaatctgaaaataaagaaaaattacttcctaatggttcaaggaaaaaataataattttatttttgtttataatattatgaaaatatttaaattataaaactttaatttttatttttttattgtgaaatgtataaaaaatacataaaataataaaattgtgttttagccatcctggctgttgaggccgcaaggcccgcaagcagtagccggtaaaggaaaaaccaggggcaatatttttgcagggtttttttttttttttttctttaaaagtaaagaacgtatgtatgagtcttaaagatagtaattttaatagagtctttgatcttatataattctcacacatttttacaatctgatgtggaatcctaaagtactaactcgtgtctatgcccatcactcgcaaacttcaatcaggatcacatcatggactctcattttttctttgttttcacttaagtgattaattttctttttgtcaaaggtaaagaatatacacacatattagaaacaggattagataattataaaaaaaggataattttaatgaaatttttaattctatataattcattcacacgtactttcaccgcttaatatgtgatatgaaggaatttagccctaatttggttaagaattaatataaattaaaattatattgtattagattaaattaaaataaaaatattaaattaatttttttagaaaaattaaaattgatcttgaaccaaactcaaataaagttaatttgatcccttcattttttttttattttaatgaaaatttaaattgagatcttgtaattttggaagccatttaaatattatcgatttgctaataattatgctgaatgtaatttaatggtaaagaaaataaataataaaaaagatacatttaatttaatttaatttatatatttttttatttcaaaaaaatttaaaaaggaacagattgttaaatctttatttttttaattaaattaaatttaattgagtctcaaatataatattttataatcttaaaaataattttaatattactgatttaaatttatagatttaatttaaaaatttttaaaagtaaagaaaataattaagattttaatttttaagtcgcacgtgattttgaatttaattttttaaaaacaaagactaacttatttttttataatttattaagaaaatcatgaaaatccccattctaaatcgacttctggaactgggatgatgcgtttgctttgcgatactccatgtgctttacttaccccataaggatcatgcgcgaatcacgatagaaccaatacaacagcaacacgtttacacgctccttttcttaacagctggcctgccattcccacgaatttccatctataagtagagaggtttggttttagcatcaaaccataatcggttgatagcctccatcagcgttttcagaaaggcgggtttcttttttgaaacttaagcgactgcgttttgaattttgatcttccatttttgcaaaaggaaatcttcgatt

SEQ ID NO: 4 - DNA, 919 bp, Hevea brasiliensis
aaccgtccaccaatctttgagttccagtgagtcatctactggttgcttgacagatccatcaataaaaccatatttctttttggcccgtaatgcagtcagcatagctcgcgcccattcttcgtaattctcgcccttcaactgaacttgggtaatcaagttatctgggttgtcattcgaattcagtgtttaagaactaaaagttttcttccctgatccagaactctcatttttcttttcatcaaccatggctctgataccatgtaaaaaaactaagaaattttggaataagaattcttatctttattgccccagaaataaaatatatatataaaaaaattacagctaacaaataggtccctaatcaagctaaactaccaaaattgtatcaaagtcatacaacaaaaggtaaaaacagatatgcacacaaaaattcctaaacaaatgccctaaataaatacaaaataagtgacagctaacagctgcatttccaataattaatttaactaataaaatttataatcttaaaaataattttaatattattgaattaaaatttataaataaaattaacactgttaaaattaaaagaaaattattaagatttgaatttttaagcggttatttaattttgaaaaacaaggctaacttttttttttatataatttactaaaaaattcatgaatgaaaaaaaaaaatccataagtaaacttaccccatacgggttatgcacgctaaaccaataaaacagaaacacgtttatacactcgttttcatttccatctataaatagagagatttgtttttagttttaaaccataatcagttgatagcttccacagtgttttccgaaaggcaaatcttttttcaaacttcagcgactgcgttttgaatttgtgatttttaaaggaaattttcaatt

SEQ ID NO: 5 - DNA, 1680 bp, Hevea brasiliensis
ggctaccttattgggaactaccaatttgtggattgtggtgattgaattaactaataagcaactgaatgttaatttccagaataagaaaacttgctgattgtaatctcaagttctagagtgaaaataaagataattatataaaatatatggaaattattatcctagaggaaattttatttttttttaaattaataaaatttttgtaattaaaaattttacgaaaaaaaatctaataaaataaatttatgtaaaattactttattttttataataaaataattacattatgtatgaaactaagtaatcatagaatatatatatatattatttagtttatgtgtcaaatataatagattaatattttctttattatttttcaaaataattttcatgtcaacccaattaaataaatatccaactaattttttttttaaatatttttatttcacagagaataatttgtatataaaaaataattttcataaaaatattttttattatttaattttaacattaattaatggtacgtgttcatattatatatgaataatatttttatattttaataaaattatcaaagttgagaaaatgatttgctcttttaagttctctcttaaaaaagaaagtcatttttcttaaaaataatttaatttctctttgactaaaatattttttgttaattatttttttaatactccaaacacaaaaaatgtgaaaaaaaaaatattttccacgacacaaacaaacagaattttagccaatcaattagcgcaattttcaactcccccgcctcctaaaggctggactggtgttgttcctggaggctgatatcctaagcaggtttctggatttgcactgattccatgatggttgaggcaagagggtatttctaatgagtttttatttagccctcttggttgttgcctgccactggaaatcaccatggaaacatatatgaagtcaaatgacaatttttattttttaaattttctgagagtgaggaaatgaataagaagaatttgttatttttctttaaagtcgtgttacttttacataatatattaagtcaaatttatcgactcagtgaaaataatttatattttataaataagaaaaatcttgttatataatttaatataaattttatatcttttttttttcaaggaaataaattttatatcttgatgataagatagagataagatcgagttaacccttgcgttaattggatgtttaaatgcttaatgcatggctaaggaaattaatgtctaaaataacagaaatgagaaaaataaatgaagggtgaaaaataaataaaacctggccctatgctctatattggggatggagtgggagccacctaatgtgtcagtgttcatcttcgaacaacgactcgattcaaagcacacccatgaagccgcttcacatcatccctttgaaactttccaccctaatcagctatcacacgatctactttccaatctcatcaacgctccaaatctcaccaccattcagtccactttcacttcctccttgtcctaatcatctttaatccatcggggtattatggtaattacatgatcaagtctctctgctataaataaagccaagtgagcttagctcatcatcacatcatttgcataccagaaaatcaagaattgggaagaaatgggaagagtt

SEQ ID NO: 6 - DNA, 1610 bp, Hevea brasiliensis
taccagctatgattcacctctagtgatattgattttattaaaaattaaggcaatgatgaatttctttttgaaaaaatcatttaagattcaagagggagatacagtgatgtcgttattttttaattttatgtaagtaaaattcgtcaatcattcatcaaagttaactgcgtgctaaataatttaaaaattattgttttttatttttgaaaattataataaaattcatttgttttaataattaggttcttagtttataatttttttattttaaatttaagtatttatgattaattctgatttaatttctgataattttaaaattaaaattatttgattcttacaaatttttaacaatcattgttttagaccaatctcaaagtaaatgtttcacacgttacaagggtgcaaaatgattggacggtgacagaaacagtaaatattatgaatttaattgttgccatgggctgctaaattcaaagggtcatcattacgtgattctcgatttacgaaaaaaaaaaagtattttcatatatatatgtatatacacacacacatcatgcaaaatatttagttaataattttccaaaattaaaacttttttttatagcatacaattaaaatgttaaattcaattaaaaaagtgaaaataaaaatataattttttacataaaaaatataaattttatataattattagtgagaatatatattactagatttaaaatatactgaataaccactcgctttttaattggttatagtgattaattaagaattttttttatctaaatttattaagtgatccaacaaattttgaactattatataagtttataaaattttgattctccattctacatttttaaattttcattttttatattatgaaaatatatacataaaaaaattaattaaactagagttaattgtcagaatgaatctctagtaaaattttctctgattaaaaaataaatttcataaattatcccactaaacttttgtcatgtgatcatgtccccaataaaatttgattttattataattggcaactcgatgtctaacctgcgagtaattatacaccatccccatgatacctccatgatttcaagtgtcaaagtatgttttaatgagaaattattaggttaactcaatgtatatacattattttttataattatgtgaaattaattctcataattatataggacacatacttcgtccacttattttttagaaaaaaagcattattttttagcactttcaatgtaactaataattaacggtttttaacatgtaagtataattgaatattataaaacgcattaatacatatatatgcatgattcttgttaatttaccattctacgtagaatattccatatagaatcaatgctttattatataataatttctgctacataataagaggctttcatttcctttgtctttaaataaccccaagtctcacttgtaaaccaacgtcgctcatttatccctcttaccctgtccctctccaactctcaaactttctggaattccatagattgtggaaactctctagctaaaccaaaaaacagaaaagaacatacaaaattgaaatactaaggtgc

SEQ ID NO: 7 - DNA, 783 bp, Solanum lycopersicum
atgtctgctcgtggactcaacaagatttcatgctcactcaacttacaaaccgaaaagctttgttatgaggataatgataatgatcttgatgaagaacttatgcctaaacacattgctttgataatggatggtaataggagatgggcaaaggataagggtttagaagtatatgaaggtcacaaacatattattccaaaattaaaagagatttgtgacatttcttctaaattgggaatacaaattatcactgcttttgcattctctactgaaaattggaaacgatccaaggaggaggttgatttcttgttgcaaatgttcgaagaaatctatgatgagttttcgaggtctggagtaagagtgtctattataggttgtaaatccgacctcccaatgacattacaaaaatgcatagcattaacagaagagactacaaagggcaacaaaggacttcaccttgtgattgcactaaactatggtggatattatgacatattgcaagcaacaaaaagcattgttaataaagcaatgaatggtttattagatgtagaagatatcaacaagaatttatttgatcaagaacttgaaagcaagtgtccaaatcctgatttacttataaggacaggaggtgaacaaagagttagtaactttttgttgtggcaattggcttacactgaattttacttcaccaacacattgtttcctgattttggagaggaagatcttaaagaggcaataatgaactttcaacaaaggcatagacgttttggtggacacacatattga

SEQ ID NO: 8 - protein, 260 aa, Solanum lycopersicum
MSARGLNKISCSLNLQTEKLCYEDNDNDLDEELMPKHIALIMDGNRRWAKDKGLEVYEGHKHIIPKLKEICDISSKLGIQIITAFAFSTENWKRSKEEVDFLLQMFEEIYDEFSRSGVRVSIIGCKSDLPMTLQKCIALTEETTKGNKGLHLVIALNYGGYYDILQATKSIVNKAMNGLLDVEDINKNLFDQELESKCPNPDLLIRTGGEQRVSNFLLWQLAYTEFYFTNTLFPDFGEEDLKEAIMNFQQRHRRFGGHTY

SEQ ID NO: 9 - DNA, 39 bp, Artificial Sequence
  PRIMER-1
ctgtattttcagggcggatattctgctcgtggactcaac

SEQ ID NO: 10 - DNA, 37 bp, Artificial Sequence
  PRIMER-2
caaaactagtgcggccgcgtcaatatgtgtgtccacc

SEQ ID NO: 11 - DNA, 792 bp, Solanum lycopersicum
atgtctgctcgtggactcaacaagatttcatgctcactcaacttacaaaccgaaaagctttgttatgaggataatgataatgatcttgatgaagaacttatgcctaaacacattgctttgataatggatggtaataggagatgggcaaaggataagggtttagaagtatatgaaggtcacaaacatattattccaaaattaaaagagatttgtgacatttcttctaaattgggaatacaaattatcactgcttttgcattctctactgaaaattggaaacgatccaaggaggaggttgatttcttgttgagtttatttgagagatcactcaaaacagaatttcagaacttagccaagaacaatgttcggataattataggttgtaaatccgacctcccaatgacattacaaaaatgcatagcattaacagaagagactacaaagggcaacaaaggacttcaccttgtgattgcactaaactatggtggatattatgacatattgcaagcaacaaaaagcattgttaataaagcaatgaatggtttattagatgtagaagatatcaacaagaatttatttgatcaagaacttgaaagcaagtgtccaaatcctgatttacttataaggacaggaggtgaacaaagagttagtaactttttgttgtggcaattggcttacactgaattttacttcaccaacacattgtttcctgattttggagaggaagatcttaaagaggcaataatgaactttcaacaaaggcatagacgttttggtggacacacatattga

SEQ ID NO: 12 - protein, 263 aa, Solanum lycopersicum
MSARGLNKISCSLNLQTEKLCYEDNDNDLDEELMPKHIALIMDGNRRWAKDKGLEVYEGHKHIIPKLKEICDISSKLGIQIITAFAFSTENWKRSKEEVDFLLSLFERSLKTEFQNLAKNNVRIIIGCKSDLPMTLQKCIALTEETTKGNKGLHLVIALNYGGYYDILQATKSIVNKAMNGLLDVEDINKNLFDQELESKCPNPDLLIRTGGEQRVSNFLLWQLAYTEFYFTNTLFPDFGEEDLKEAIMNFQQRHRRFGGHTY

SEQ ID NO: 13 - protein, 21 aa, Arabidopsis thaliana
SLFERSLKTEFQNLAKNNVRI

SEQ ID NO: 14 - protein, 21 aa, Escherichia coli
ELFVWALDSEVKSLHRHNVRL

SEQ ID NO: 15 - protein, 21 aa, Micrococcus luteus
KLPGDFLNTFLPELIEKNVKV

SEQ ID NO: 16 - protein, 26 aa, Saccharomyces cerevisiae
NLFTVKLDEFAKRAKDYKDPLYGSKI

SEQ ID NO: 17 - protein, 24 aa, Homo sapiens
DLARQKFSRLMEEKEKLQKHGVCI

SEQ ID NO: 18 - DNA, 804 bp, Solanum lycopersicum
atgtctgctcgtggactcaacaagatttcatgctcactcaacttacaaaccgaaaagctttgttatgaggataatgataatgatcttgatgaagaacttatgcctaaacacattgctttgataatggatggtaataggagatgggcaaaggataagggtttagaagtatatgaaggtcacaaacatattattccaaaattaaaagagatttgtgacatttcttctaaattgggaatacaaattatcactgcttttgcattctctactgaaaattggaaacgatccaaggaggaggttcagtacgtaatggatctaatgctggagaagattgaagggatgatcatggaagaaagtatcatcaatgcatatgatatttgcgtatctattataggttgtaaatccgacctcccaatgacattacaaaaatgcatagcattaacagaagagactacaaagggcaacaaaggacttcaccttgtgattgcactaaactatggtggatattatgacatattgcaagcaacaaaaagcattgttaataaagcaatgaatggtttattagatgtagaagatatcaacaagaatttatttgatcaagaacttgaaagcaagtgtccaaatcctgatttacttataaggacaggaggtgaacaaagagttagtaactttttgttgtggcaattggcttacactgaattttacttcaccaacacattgtttcctgattttggagaggaagatcttaaagaggcaataatgaactttcaacaaaggcatagacgttttggtggacacacatattga

SEQ ID NO: 19 - protein, 267 aa, Solanum lycopersicum
MSARGLNKISCSLNLQTEKLCYEDNDNDLDEELMPKHIALIMDGNRRWAKDKGLEVYEGHKHIIPKLKEICDISSKLGIQIITAFAFSTENWKRSKEEVQYVMDLMLEKIEGMIMEESIINAYDICVSIIGCKSDLPMTLQKCIALTEETTKGNKGLHLVIALNYGGYYDILQATKSIVNKAMNGLLDVEDINKNLFDQELESKCPNPDLLIRTGGEQRVSNFLLWQLAYTEFYFTNTLFPDFGEEDLKEAIMNFQQRHRRFGGHTY

SEQ ID NO: 20 - DNA, 34 bp, Artificial Sequence
  PRIMER-3
tttggatccgatggaattatacaacggtgagagg

SEQ ID NO: 21 - DNA, 39 bp, Artificial Sequence
  PRIMER-4
tttgcggccgcttattttaagtattccttatgtttctcc

SEQ ID NO: 22 - DNA, 873 bp, Hevea brasiliensis
atggaattatacaacggtgagaggccaagtgtgttcagacttttagggaagtatatgagaaaagggttatatagcatcctaacccagggtcccatccctactcatattgccttcatattggatggaaacaggaggtttgctaagaagcataaactgccagaaggaggtggtcataaggctggatttttagctcttctgaacgtactaacttattgctatgagttaggagtgaaatatgcgactatctatgcctttagcatcgataattttcgaaggaaacctcatgaggttcagtacgtaatggatctaatgctggagaagattgaagggatgatcatggaagaaagtatcatcaatgcatatgatatttgcgtacgttttgtgggtaacctgaagcttttaagtgagccagtcaagaccgcagcagataagattatgagggctactgccaacaattccaaatgtgtgcttctcattgctgtatgctatacttcaactgatgagatcgtgcatgctgttgaagaatcctctgaattgaactccaatgaagtttgtaacaatcaagaattggaggaggcaaatgcaactggaagcggtactgtgattcaaattgagaacatggagtcgtattctggaataaaacttgtagaccttgagaaaaacacctacataaatccttatcctgatgttctgattcgaacttctggggagacccgtctgagcaactacttactttggcagactactaattgcatactgtattctcctcatgcactgtggccagagattggtcttcgacacgtggtgtgggcagtaattaacttccaacgtcattattcttacttggagaaacataaggaatacttaaaataa

SEQ ID NO: 23 - protein, 290 aa, Hevea brasiliensis
MELYNGERPSVFRLLGKYMRKGLYSILTQGPIPTHIAFILDGNRRFAKKHKLPEGGGHKAGFLALLNVLTYCYELGVKYATIYAFSIDNFRRKPHEVQYVMDLMLEKIEGMIMEESIINAYDICVRFVGNLKLLSEPVKTAADKIMRATANNSKCVLLIAVCYTSTDEIVHAVEESSELNSNEVCNNQELEEANATGSGTVIQIENMESYSGIKLVDLEKNTYINPYPDVLIRTSGETRLSNYLLWQTTNCILYSPHALWPEIGLRHVVWAVINCQRHYSYLEKHKEYLK

SEQ ID NO: 24 - protein, 24 aa, Hevea brasiliensis
DLMLEKIEGMIMEESIINAYDICV